European Patent Application EP 4 756 028 A2, published June 10, 2026. Title: Pharmaceutical compositions for treatment of microRNA related diseases. Applicant: F. Hoffmann-La Roche AG. The sequence listing filed with the application follows.

SEQUENCE LISTING (8 sequences)

SEQ ID NO: 1 - RNA, 22 nt, Homo sapiens
  source 1..22: mol_type = other RNA
tgtgactggttgaccagagggg

SEQ ID NO: 2 - DNA, 1273 bp, Homo sapiens
  source 1..1273: mol_type = other DNA
ggaccacaatttcaactccagggaagggggactgtgccagcaccactccaagggaggtgagtgaagggttgcccaaactccagtgtgttcctaggacacccgtaagctgcctcactaatgctcggtgtccactctgtccacaggatggtggttggcagccactccccttggagaagtggaaggggactccttgtctgtcttgtctctgcttttctgtggtacttgaagagaagttgttcgtggtggattcgctttacttatgacgaatcattcacggacaacacttttttcagtaccaaatgctacctctaaggacttcctggacacaatggcagcttcaggaaagatagtctttgtgtcaaccatgtggaaaagccaagaatggatggcgggccatggacaatgcgctgacctagctgtaagtcacctggcccgataatccgagcctcccatgcacctataggaggtcttcccatgggtctcaccaactctggggaatcagctgtggttctgtcaccagcgtcacctcacaagactttgaagagaggctccctgggccccaggccgacttccagaagagatgttggtgtcagcaccgtccagggtgtgtgactggttgaccagaggggcatgcactgtgttcaccctgtgggccacctagtcaccaaccctcagcatcactcccactccaggaagactttccagagctcccaccaactctggggaagcggccatggacttgctgtgactgcttggtggactgcgatgacacgtgctcttgggggtgtatgtttacttaaaatgcaatgagtcagccttggcagccccttcaccactgtgacagcctccttgaagtgttgacttccgatgtgggacgccatgttgtcttctgttgagggacctgatgtgggccagcttttctcctgggtgtgtgactgaatccttcttcccagagcatgtgctgcctttgttaggtctgtcacgtcgtcctctaatacccagcatcctgtctctccctaggaggctccatggagataatgcggctttgggaagcggccatgattctcctgtcagggaccagtgagctacgcaaaagctccctgtcttgtctggaaggacgaactgcatccttgctgctggggagaaggcagtgccctcagcactcccttaaggtaagtgcgcctcgggtgagcatgcacttaatgtgggtgtatgtcactcggctcggcccactacccaatactatcccacccattcctaacaggactcccga

SEQ ID NO: 3 - DNA, 73 bp, Homo sapiens
  source 1..73: mol_type = other DNA
cagggtgtgtgactggttgaccagaggggcatgcactgtgttcaccctgtgggccacctagtcaccaaccctc

SEQ ID NO: 4 - RNA, 31 nt, Homo sapiens
  source 1..31: mol_type = other RNA
tctctccctctggtcaaccagtcacaaggct

SEQ ID NO: 5 - DNA, 22 bp, synthetic construct
  misc_feature 1..22: note = Oligonucleotide base sequence
  source 1..22: mol_type = other DNA
cccctctggtcaaccagtcaca

SEQ ID NO: 6 - DNA, 15 bp, synthetic construct
  misc_feature 1..15: note = Oligonucleotide base sequence
  source 1..15: mol_type = other DNA
cgtctagccacctag

SEQ ID NO: 7 - DNA, 19 bp, synthetic construct
  misc_feature 1..19: note = Oligonucleotide base sequence
  source 1..19: mol_type = other DNA
cctctggtcaaccagtcac

SEQ ID NO: 8 - DNA, 15 bp, synthetic construct
  misc_feature 1..15: note = Oligonucleotide base sequence
  source 1..15: mol_type = other DNA
tggtcaaccagtcac